European Patent Application EP 4 545 546 A1, published April 30, 2025. Title: INSECT NEUROPEPTIDES 8. Applicant: SOLASTA Bio Limited. The sequence listing filed with the application follows.

SEQUENCE LISTING (16 sequences)

SEQ ID NO: 1 - protein, 9 aa, synthetic construct
  source 1..9: note = Z peptide
LTFTSSWGG

SEQ ID NO: 2 - protein, 9 aa, synthetic construct
  source 1..9: note = SB-P-86
  MOD_RES 9: note = glycinamide
  MOD_RES 1: note = pyroglutamyl-leucine
LTFTSSWGG

SEQ ID NO: 3 - protein, 11 aa, synthetic construct
  source 1..11: note = SB-P-47
  MOD_RES 11: note = leucinamide
  MOD_RES 1: note = pyroglutamyl-alanine
AIMARPQVPRL

SEQ ID NO: 4 - protein, 8 aa, synthetic construct
  source 1..8: note = SB-P-49
  MOD_RES 8: note = leucinamide
SVPFKPRL

SEQ ID NO: 5 - protein, 19 aa, synthetic construct
  source 1..19: note = SB-P-51
  MOD_RES 19: note = leucinamide
LRQLQSNGEPAYRVRTPRL

SEQ ID NO: 6 - protein, 16 aa, synthetic construct
  source 1..16: note = SB-P-80
  MOD_RES 16: note = leucinamide
NADEDQQQSVDFTPRL

SEQ ID NO: 7 - protein, 10 aa, synthetic construct
  source 1..10: note = SB-P-81
  MOD_RES 10: note = leucinamide
GGSMTFSPRL

SEQ ID NO: 8 - protein, 8 aa, synthetic construct
  source 1..8: note = SB-P-70
  MOD_RES 8: note = glycinamide
KVKFSAWG

SEQ ID NO: 9 - protein, 10 aa, synthetic construct
  source 1..10: note = SB-P-65
  MOD_RES 10: note = glycinamide
RQKTVFSSWG

SEQ ID NO: 10 - protein, 7 aa, synthetic construct
  source 1..7: note = SB-P-66
  MOD_RES 7: note = glycinamide
PAFSSWG

SEQ ID NO: 11 - protein, 12 aa, synthetic construct
  source 1..12: note = SB-P-46
  MOD_RES 12: note = leucinamide
SPPYSPPFSPRL

SEQ ID NO: 12 - protein, 8 aa, synthetic construct
  source 1..8: note = SB-P-039
  MOD_RES 1: note = palmitoyl-glutamine
  MOD_RES 8: note = tryptophanamide
QLTFSPDW

SEQ ID NO: 13 - protein, 7 aa, synthetic construct
  source 1..7: note = SB-P-042
  MOD_RES 1: note = pyroglutamyl-leucine
  MOD_RES 7: note = tryptophanamide
LTFSPDW

SEQ ID NO: 14 - protein, 6 aa, synthetic construct
  source 1..6: note = SB-P-69
  MOD_RES 6: note = glycinamide
NFSPWG

SEQ ID NO: 15 - protein, 19 aa, synthetic construct
  source 1..19: note = SB-P-48
  MOD_RES 19: note = leucinamide
EQNVQSNGEPAYRVRTPRL

SEQ ID NO: 16 - protein, 8 aa, synthetic construct
  source 1..8: note = SB-P-41
  MOD_RES 8: note = tryptophanamide
QLTFSPDW